European Patent Application EP 4 806 450 A1, published September 16, 2026. Title: NOVEL PEPTIDES WITH SPECIFICITY FOR THE HEART. Applicant: Universitaetsklinikum Hamburg-Eppendorf. Application EP. The sequence listing filed with the application follows.

SEQUENCE LISTING (12 sequences)

SEQ ID NO: 1 - protein, 6 aa, synthetic construct
DWPATY

SEQ ID NO: 2 - protein, 6 aa, synthetic construct
DWPQSM

SEQ ID NO: 3 - protein, 6 aa, synthetic construct
DWPQDL

SEQ ID NO: 4 - protein, 735 aa, Adeno-associated dependoparvovirus A [sequence omitted]

SEQ ID NO: 5 - protein, 598 aa, Adeno-associated dependoparvovirus A
MAPGKKRPVEHSPVEPDSSSGTGKAGQQPARKRLNFGQTGDADSVPDPQPLGQPPAAPSGLGTNTMATGSGAPMADNNEGADGVGNSSGNWHCDSTWMGDRVITTSTRTWALPTYNNHLYKQISSQSGASNDNHYFGYSTPWGYFDFNRFHCHFSPRDWQRLINNNWGFRPKRLNFKLFNIQVKEVTQNDGTTTIANNLTSTVQVFTDSEYQLPYVLGSAHQGCLPPFPADVFMVPQYGYLTLNNGSQAVGRSSFYCLEYFPSQMLRTGNNFTFSYTFEDVPFHSSYAHSQSLDRLMNPLIDQYLYYLSRTNTPSGTTTQSRLQFSQAGASDIRDQSRNWLPGPCYRQQRVSKTSADNNNSEYSWTGATKYHLNGRDSLVNPGPAMASHKDDEEKFFPQSGVLIFGKQGSEKTNVDIEKVMITDEEEIRTTNPVATEQYGSVSTNLQRGNRQAATADVNTQGVLPGMVWQDRDVYLQGPIWAKIPHTDGHFHPSPLMGGFGLKHPPPQILIKNTPVPANPSTTFSAAKFASFITQYSTGQVSVEIEWELQKENSKRWNPEIQYTSNYNKSVNVDFTVDTNGVYSEPRPIGTRYLTRNL

SEQ ID NO: 6 - protein, 533 aa, Adeno-associated dependoparvovirus A
MATGSGAPMADNNEGADGVGNSSGNWHCDSTWMGDRVITTSTRTWALPTYNNHLYKQISSQSGASNDNHYFGYSTPWGYFDFNRFHCHFSPRDWQRLINNNWGFRPKRLNFKLFNIQVKEVTQNDGTTTIANNLTSTVQVFTDSEYQLPYVLGSAHQGCLPPFPADVFMVPQYGYLTLNNGSQAVGRSSFYCLEYFPSQMLRTGNNFTFSYTFEDVPFHSSYAHSQSLDRLMNPLIDQYLYYLSRTNTPSGTTTQSRLQFSQAGASDIRDQSRNWLPGPCYRQQRVSKTSADNNNSEYSWTGATKYHLNGRDSLVNPGPAMASHKDDEEKFFPQSGVLIFGKQGSEKTNVDIEKVMITDEEEIRTTNPVATEQYGSVSTNLQRGNRQAATADVNTQGVLPGMVWQDRDVYLQGPIWAKIPHTDGHFHPSPLMGGFGLKHPPPQILIKNTPVPANPSTTFSAAKFASFITQYSTGQVSVEIEWELQKENSKRWNPEIQYTSNYNKSVNVDFTVDTNGVYSEPRPIGTRYLTRNL

SEQ ID NO: 7 - protein, 743 aa, synthetic construct
MAADGYLPDWLEDTLSEGIRQWWKLKPGPPPPKPAERHKDDSRGLVLPGYKYLGPFNGLDKGEPVNEADAAALEHDKAYDRQLDSGDNPYLKYNHADAEFQERLKEDTSFGGNLGRAVFQAKKRVLEPLGLVEEPVKTAPGKKRPVEHSPVEPDSSSGTGKAGQQPARKRLNFGQTGDADSVPDPQPLGQPPAAPSGLGTNTMATGSGAPMADNNEGADGVGNSSGNWHCDSTWMGDRVITTSTRTWALPTYNNHLYKQISSQSGASNDNHYFGYSTPWGYFDFNRFHCHFSPRDWQRLINNNWGFRPKRLNFKLFNIQVKEVTQNDGTTTIANNLTSTVQVFTDSEYQLPYVLGSAHQGCLPPFPADVFMVPQYGYLTLNNGSQAVGRSSFYCLEYFPSQMLRTGNNFTFSYTFEDVPFHSSYAHSQSLDRLMNPLIDQYLYYLSRTNTPSGTTTQSRLQFSQAGASDIRDQSRNWLPGPCYRQQRVSKTSADNNNSEYSWTGATKYHLNGRDSLVNPGPAMASHKDDEEKFFPQSGVLIFGKQGSEKTNVDIEKVMITDEEEIRTTNPVATEQYGSVSTNLQRGQRGDWPATYAQAATADVNTQGVLPGMVWQDRDVYLQGPIWAKIPHTDGHFHPSPLMGGFGLKHPPPQILIKNTPVPANPSTTFSAAKFASFITQYSTGQVSVEIEWELQKENSKRWNPEIQYTSNYNKSVNVDFTVDTNGVYSEPRPIGTRYLTRNL

SEQ ID NO: 8 - protein, 743 aa, synthetic construct
MAADGYLPDWLEDTLSEGIRQWWKLKPGPPPPKPAERHKDDSRGLVLPGYKYLGPFNGLDKGEPVNEADAAALEHDKAYDRQLDSGDNPYLKYNHADAEFQERLKEDTSFGGNLGRAVFQAKKRVLEPLGLVEEPVKTAPGKKRPVEHSPVEPDSSSGTGKAGQQPARKRLNFGQTGDADSVPDPQPLGQPPAAPSGLGTNTMATGSGAPMADNNEGADGVGNSSGNWHCDSTWMGDRVITTSTRTWALPTYNNHLYKQISSQSGASNDNHYFGYSTPWGYFDFNRFHCHFSPRDWQRLINNNWGFRPKRLNFKLFNIQVKEVTQNDGTTTIANNLTSTVQVFTDSEYQLPYVLGSAHQGCLPPFPADVFMVPQYGYLTLNNGSQAVGRSSFYCLEYFPSQMLRTGNNFTFSYTFEDVPFHSSYAHSQSLDRLMNPLIDQYLYYLSRTNTPSGTTTQSRLQFSQAGASDIRDQSRNWLPGPCYRQQRVSKTSADNNNSEYSWTGATKYHLNGRDSLVNPGPAMASHKDDEEKFFPQSGVLIFGKQGSEKTNVDIEKVMITDEEEIRTTNPVATEQYGSVSTNLQRGQRGDWPQSMAQAATADVNTQGVLPGMVWQDRDVYLQGPIWAKIPHTDGHFHPSPLMGGFGLKHPPPQILIKNTPVPANPSTTFSAAKFASFITQYSTGQVSVEIEWELQKENSKRWNPEIQYTSNYNKSVNVDFTVDTNGVYSEPRPIGTRYLTRNL

SEQ ID NO: 9 - protein, 743 aa, synthetic construct
MAADGYLPDWLEDTLSEGIRQWWKLKPGPPPPKPAERHKDDSRGLVLPGYKYLGPFNGLDKGEPVNEADAAALEHDKAYDRQLDSGDNPYLKYNHADAEFQERLKEDTSFGGNLGRAVFQAKKRVLEPLGLVEEPVKTAPGKKRPVEHSPVEPDSSSGTGKAGQQPARKRLNFGQTGDADSVPDPQPLGQPPAAPSGLGTNTMATGSGAPMADNNEGADGVGNSSGNWHCDSTWMGDRVITTSTRTWALPTYNNHLYKQISSQSGASNDNHYFGYSTPWGYFDFNRFHCHFSPRDWQRLINNNWGFRPKRLNFKLFNIQVKEVTQNDGTTTIANNLTSTVQVFTDSEYQLPYVLGSAHQGCLPPFPADVFMVPQYGYLTLNNGSQAVGRSSFYCLEYFPSQMLRTGNNFTFSYTFEDVPFHSSYAHSQSLDRLMNPLIDQYLYYLSRTNTPSGTTTQSRLQFSQAGASDIRDQSRNWLPGPCYRQQRVSKTSADNNNSEYSWTGATKYHLNGRDSLVNPGPAMASHKDDEEKFFPQSGVLIFGKQGSEKTNVDIEKVMITDEEEIRTTNPVATEQYGSVSTNLQRGQRGDWPQDLAQAATADVNTQGVLPGMVWQDRDVYLQGPIWAKIPHTDGHFHPSPLMGGFGLKHPPPQILIKNTPVPANPSTTFSAAKFASFITQYSTGQVSVEIEWELQKENSKRWNPEIQYTSNYNKSVNVDFTVDTNGVYSEPRPIGTRYLTRNL

SEQ ID NO: 10 - DNA, 2232 bp, synthetic construct
  source 1..2232: mol_type = other DNA
atggctgccgatggttatcttccagattggctcgaggacactctctctgaaggaataagacagtggtggaagctcaaacctggcccaccaccaccaaagcccgcagagcggcataaggacgacagcaggggtcttgtgcttcctgggtacaagtacctcggacccttcaacggactcgacaagggagagccggtcaacgaggcagacgccgcggccctcgagcacgacaaagcctacgaccggcagctcgacagcggagacaacccgtacctcaagtacaaccacgccgacgcggagtttcaggagcgccttaaagaagatacgtcttttgggggcaacctcggacgagcagtcttccaggcgaaaaagagggttcttgaacctctgggcctggttgaggaacctgttaagacggctccgggaaaaaagaggccggtagagcactctcctgtggagccagactcctcctcgggaaccggaaaggcgggccagcagcctgcaagaaaaagattgaattttggtcagactggagacgcagactcagtacctgacccccagcctctcggacagccaccagcagccccctctggtctgggaactaatacgatggctacaggcagtggcgcaccaatggcagacaataacgagggcgccgacggagtgggtaattcctcgggaaattggcattgcgattccacatggatgggcgacagagtcatcaccaccagcacccgaacctgggccctgcccacctacaacaaccacctctacaaacaaatttccagccaatcaggagcctcgaacgacaatcactactttggctacagcaccccttgggggtattttgacttcaacagattccactgccacttttcaccacgtgactggcaaagactcatcaacaacaactggggattccgacccaagagactcaacttcaagctctttaacattcaagtcaaagaggtcacgcagaatgacggtacgacgacgattgccaataaccttaccagcacggttcaggtgtttactgactcggagtaccagctcccgtacgtcctcggctcggcgcatcaaggatgcctcccgccgttcccagcagacgtcttcatggtgccacagtatggatacctcaccctgaacaacgggagtcaggcagtaggacgctcttcattttactgcctggagtactttccttctcagatgctgcgtaccggaaacaactttaccttcagctacacttttgaggacgttcctttccacagcagctacgctcacagccagagtctggaccgtctcatgaatcctctcatcgaccagtacctgtattacttgagcagaacaaacactccaagtggaaccaccacgcagtcaaggcttcagttttctcaggccggagcgagtgacattcgggaccagtctaggaactggcttcctggaccctgttaccgccagcagcgagtatcaaagacatctgcggataacaacaacagtgaatactcgtggactggagctaccaagtaccacctcaatggcagagactctctggtgaatccgggcccggccatggcaagccacaaggacgatgaagaaaagttttttcctcagagcggggttctcatctttgggaagcaaggctcagagaaaacaaatgtggacattgaaaaggtcatgattacagacgaagaggaaatcaggacaaccaatcccgtggctacggagcagtatggttctgtatctaccaacctccagagaggccagagaggcgactggccagctacttacgcccaggcggccaccgcagatgtcaacacacaaggcgttcttccaggcatggtctggcaggacagagatgtgtaccttcaggggcccatctgggcaaagattccacacacggacggacattttcacccctctcccctcatgggtggattcggacttaaacaccctcctccacagattctcatcaagaacaccccggtacctgcgaatccttcgaccaccttcagtgcggcaaagtttgcttccttcatcacacagtactccacgggacaggtcagcgtggagatcgagtgggagctgcagaaggaaaacagcaaacgctggaatcccgaaattcagtacacttccaactacaacaagtctgttaatgtggactttactgtggacactaatggcgtgtattcagagcctcgccccattggcaccagatacctgactcgtaatctgtaa

SEQ ID NO: 11 - DNA, 2232 bp, synthetic construct
  source 1..2232: mol_type = other DNA
atggctgccgatggttatcttccagattggctcgaggacactctctctgaaggaataagacagtggtggaagctcaaacctggcccaccaccaccaaagcccgcagagcggcataaggacgacagcaggggtcttgtgcttcctgggtacaagtacctcggacccttcaacggactcgacaagggagagccggtcaacgaggcagacgccgcggccctcgagcacgacaaagcctacgaccggcagctcgacagcggagacaacccgtacctcaagtacaaccacgccgacgcggagtttcaggagcgccttaaagaagatacgtcttttgggggcaacctcggacgagcagtcttccaggcgaaaaagagggttcttgaacctctgggcctggttgaggaacctgttaagacggctccgggaaaaaagaggccggtagagcactctcctgtggagccagactcctcctcgggaaccggaaaggcgggccagcagcctgcaagaaaaagattgaattttggtcagactggagacgcagactcagtacctgacccccagcctctcggacagccaccagcagccccctctggtctgggaactaatacgatggctacaggcagtggcgcaccaatggcagacaataacgagggcgccgacggagtgggtaattcctcgggaaattggcattgcgattccacatggatgggcgacagagtcatcaccaccagcacccgaacctgggccctgcccacctacaacaaccacctctacaaacaaatttccagccaatcaggagcctcgaacgacaatcactactttggctacagcaccccttgggggtattttgacttcaacagattccactgccacttttcaccacgtgactggcaaagactcatcaacaacaactggggattccgacccaagagactcaacttcaagctctttaacattcaagtcaaagaggtcacgcagaatgacggtacgacgacgattgccaataaccttaccagcacggttcaggtgtttactgactcggagtaccagctcccgtacgtcctcggctcggcgcatcaaggatgcctcccgccgttcccagcagacgtcttcatggtgccacagtatggatacctcaccctgaacaacgggagtcaggcagtaggacgctcttcattttactgcctggagtactttccttctcagatgctgcgtaccggaaacaactttaccttcagctacacttttgaggacgttcctttccacagcagctacgctcacagccagagtctggaccgtctcatgaatcctctcatcgaccagtacctgtattacttgagcagaacaaacactccaagtggaaccaccacgcagtcaaggcttcagttttctcaggccggagcgagtgacattcgggaccagtctaggaactggcttcctggaccctgttaccgccagcagcgagtatcaaagacatctgcggataacaacaacagtgaatactcgtggactggagctaccaagtaccacctcaatggcagagactctctggtgaatccgggcccggccatggcaagccacaaggacgatgaagaaaagttttttcctcagagcggggttctcatctttgggaagcaaggctcagagaaaacaaatgtggacattgaaaaggtcatgattacagacgaagaggaaatcaggacaaccaatcccgtggctacggagcagtatggttctgtatctaccaacctccagagaggccagagaggcgactggccacagtctatggcccaggcggccaccgcagatgtcaacacacaaggcgttcttccaggcatggtctggcaggacagagatgtgtaccttcaggggcccatctgggcaaagattccacacacggacggacattttcacccctctcccctcatgggtggattcggacttaaacaccctcctccacagattctcatcaagaacaccccggtacctgcgaatccttcgaccaccttcagtgcggcaaagtttgcttccttcatcacacagtactccacgggacaggtcagcgtggagatcgagtgggagctgcagaaggaaaacagcaaacgctggaatcccgaaattcagtacacttccaactacaacaagtctgttaatgtggactttactgtggacactaatggcgtgtattcagagcctcgccccattggcaccagatacctgactcgtaatctgtaa

SEQ ID NO: 12 - DNA, 2232 bp, synthetic construct
  source 1..2232: mol_type = other DNA
atggctgccgatggttatcttccagattggctcgaggacactctctctgaaggaataagacagtggtggaagctcaaacctggcccaccaccaccaaagcccgcagagcggcataaggacgacagcaggggtcttgtgcttcctgggtacaagtacctcggacccttcaacggactcgacaagggagagccggtcaacgaggcagacgccgcggccctcgagcacgacaaagcctacgaccggcagctcgacagcggagacaacccgtacctcaagtacaaccacgccgacgcggagtttcaggagcgccttaaagaagatacgtcttttgggggcaacctcggacgagcagtcttccaggcgaaaaagagggttcttgaacctctgggcctggttgaggaacctgttaagacggctccgggaaaaaagaggccggtagagcactctcctgtggagccagactcctcctcgggaaccggaaaggcgggccagcagcctgcaagaaaaagattgaattttggtcagactggagacgcagactcagtacctgacccccagcctctcggacagccaccagcagccccctctggtctgggaactaatacgatggctacaggcagtggcgcaccaatggcagacaataacgagggcgccgacggagtgggtaattcctcgggaaattggcattgcgattccacatggatgggcgacagagtcatcaccaccagcacccgaacctgggccctgcccacctacaacaaccacctctacaaacaaatttccagccaatcaggagcctcgaacgacaatcactactttggctacagcaccccttgggggtattttgacttcaacagattccactgccacttttcaccacgtgactggcaaagactcatcaacaacaactggggattccgacccaagagactcaacttcaagctctttaacattcaagtcaaagaggtcacgcagaatgacggtacgacgacgattgccaataaccttaccagcacggttcaggtgtttactgactcggagtaccagctcccgtacgtcctcggctcggcgcatcaaggatgcctcccgccgttcccagcagacgtcttcatggtgccacagtatggatacctcaccctgaacaacgggagtcaggcagtaggacgctcttcattttactgcctggagtactttccttctcagatgctgcgtaccggaaacaactttaccttcagctacacttttgaggacgttcctttccacagcagctacgctcacagccagagtctggaccgtctcatgaatcctctcatcgaccagtacctgtattacttgagcagaacaaacactccaagtggaaccaccacgcagtcaaggcttcagttttctcaggccggagcgagtgacattcgggaccagtctaggaactggcttcctggaccctgttaccgccagcagcgagtatcaaagacatctgcggataacaacaacagtgaatactcgtggactggagctaccaagtaccacctcaatggcagagactctctggtgaatccgggcccggccatggcaagccacaaggacgatgaagaaaagttttttcctcagagcggggttctcatctttgggaagcaaggctcagagaaaacaaatgtggacattgaaaaggtcatgattacagacgaagaggaaatcaggacaaccaatcccgtggctacggagcagtatggttctgtatctaccaacctccagagaggccagagaggcgactggccacaggacctggcccaggcggccaccgcagatgtcaacacacaaggcgttcttccaggcatggtctggcaggacagagatgtgtaccttcaggggcccatctgggcaaagattccacacacggacggacattttcacccctctcccctcatgggtggattcggacttaaacaccctcctccacagattctcatcaagaacaccccggtacctgcgaatccttcgaccaccttcagtgcggcaaagtttgcttccttcatcacacagtactccacgggacaggtcagcgtggagatcgagtgggagctgcagaaggaaaacagcaaacgctggaatcccgaaattcagtacacttccaactacaacaagtctgttaatgtggactttactgtggacactaatggcgtgtattcagagcctcgccccattggcaccagatacctgactcgtaatctgtaa